European Patent Application EP 4 219 680 A1, published August 2, 2023. Title: NOVEL LACTIC ACID BACTERIA AND USE THEREOF. Applicant: University-Industry Cooperation Group of Kyung Hee University. The sequence listing filed with the application follows.

SEQUENCE LISTING (7 sequences)

SEQ ID NO: 1 - DNA, 1489 bp, Artificial Sequence
  Lactobacillus plantarum NK151_16SrDNA
ctcaggacgaacgctggcggcgtgcctaatacatgcaagtcgaacgaactctggtattgattggtgcttgcatcatgatttacatttgagtgagtggcgaactggtgagtaacacgtgggaaacctgcccagaagcgggggataacacctggaaacagatgctaataccgcataacaacttggaccgcatggtccgagcttgaaagatggcttcggctatcacttttggatggtcccgcggcgtattagctagatggtggggtaacggctcaccatggcaatgatacgtagccgacctgagagggtaatcggccacattgggactgagacacggcccaaactcctacgggaggcagcagtagggaatcttccacaatggacgaaagtctgatggagcaacgccgcgtgagtgaagaagggtttcggctcgtaaaactctgttgttaaagaagaacatatctgagagtaactgttcaggtattgacggtatttaaccagaaagccacggctaactacgtgccagcagccgcggtaatacgtaggtggcaagcgttgtccggatttattgggcgtaaagcgagcgcaggcggttttttaagtctgatgtgaaagccttcggctcaaccgaagaagtgcatcggaaactgggaaacttgagtgcagaagaggacagtggaactccatgtgtagcggtgaaatgcgtagatatatggaagaacaccagtggcgaaggcggctgtctggtctgtaactgacgctgaggctcgaaagtatgggtagcaaacaggattagataccctggtagtccataccgtaaacgatgaatgctaagtgttggagggtttccgcccttcagtgctgcagctaacgcattaagcattccgcctggggagtacggccgcaaggctgaaactcaaaggaattgacgggggcccgcacaagcggtggagcatgtggtttaattcgaagctacgcgaagaaccttaccaggtcttgacatactatgcaaatctaagagattagacgttcccttcggggacatggatacaggtggtgcatggttgtcgtcagctcgtgtcgtgagatgttgggttaagtcccgcaacgagcgcaacccttattatcagttgccagcattaagttgggcactctggtgagactgccggtgacaaaccggaggaaggtggggatgacgtcaaatcatcatgccccttatgacctgggctacacacgtgctacaatggatggtacaacgagttgcgaactcgcgagagtaagctaatctcttaaagccattctcagttcggattgtaggctgcaactcgcctacatgaagtcggaatcgctagtaatcgcggatcagcatgccgcggtgaatacgttcccgggccttgtacacaccgcccgtcacaccatgagagtttgtaacacccaaagtcggtggggtaaccttttaggaaccagccgcctaaggtgggacagatgatta

SEQ ID NO: 2 - DNA, 1462 bp, Artificial Sequence
  Bifidobacterium bifidum NK175_16SrDNA
ctcaggatgaacgctggcggcgtgcttaacacatgcaagtcgaacgggatccatcaagcttgcttggtggtgagagtggcgaacgggtgagtaatgcgtgaccgacctgccccatgctccggaatagctcctggaaacgggtggtaatgccggatgttccacatgatcgcatgtgattgtgggaaagattctatcggcgtgggatggggtcgcgtcctatcagcttgttggtgaggtaacggctcaccaaggcttcgacgggtagccggcctgagagggcgaccggccacattgggactgagatacggcccagactcctacgggaggcagcagtggggaatattgcacaatgggcgcaagcctgatgcagcgacgccgcgtgagggatggaggccttcgggttgtaaacctcttttgtttgggagcaagccttcgggtgagtgtacctttcgaataagcgccggctaactacgtgccagcagccgcggtaatacgtagggcgcaagcgttatccggatttattgggcgtaaagggctcgtaggcggctcgtcgcgtccggtgtgaaagtccatcgcttaacggtggatctgcgccgggtacgggcgggctggagtgcggtaggggagactggaattcccggtgtaacggtggaatgtgtagatatcgggaagaacaccgatggcgaaggcaggtctctgggccgtcactgacgctgaggagcgaaagcgtggggagcgaacaggattagataccctggtagtccacgccgtaaacggtggacgctggatgtggggcacgttccacgtgttccgtgtcggagctaacgcgttaagcgtcccgcctggggagtacggccgcaaggctaaaactcaaagaaattgacgggggcccgcacaagcggcggagcatgcggattaattcgatgcaacgcgaagaaccttacctgggcttgacatgttcccgacgacgccagagatggcgtttcccttcggggcgggttcacaggtggtgcatggtcgtcgtcagctcgtgtcgtgagatgttgggttaagtcccgcaacgagcgcaaccctcgccccgtgttgccagcacatgatggtgggaactcacgggggaccgccggggttaactcggaggaaggtggggatgacgtcagatcatcatgccccttacgtccagggcttcacgcatgctacaatggccggtacagcgggatgcgacatggcgacatggagcggatccctgaaaaccggtctcagttcggatcggagcctgcaacccggctccgtgaaggcggagtcgctagtaatcgcggatcagcaacgccgcggtgaatgcgttcccgggccttgtacacaccgcccgtcaagtcatgaaagtgggcagcacccgaagccggtggcctaaccccttgtgggatggagccgtctaaggtgaggctcgtgattgggactaagtcta

SEQ ID NO: 3 - DNA, 1460 bp, Artificial Sequence
  Bifidobacterium longum NK173_16SrDNA
ctcaggatgaacgctggcggcgtgcttaacacatgcaagtcgaacgggatccatcaagcttgcttggtggtgagagtggcgaacgggtgagtaatgcgtgaccgacctgccccatacaccggaatagctcctggaaacgggtggtaatgccggatgctccagttgatcgcatggtcttctgggaaagctttcgcggtatgggatggggtcgcgtcctatcagcttgacggcggggtaacggcccaccgtggcttcgacgggtagccggcctgagagggcgaccggccacattgggactgagatacggcccagactcctacgggaggcagcagtggggaatattgcacaatgggcgcaagcctgatgcagcgacgccgcgtgagggatggaggccttcgggttgtaaacctcttttatcggggagcaagcgagagtgagtttacccgttgaataagcaccggctaactacgtgccagcagccgcggtaatacgtagggtgcaagcgttatccggaattattgggcgtaaagggctcgtaggcggttcgtcgcgtccggtgtgaaagtccatcgcttaacggtggatccgcgccgggtacgggcgggcttgagtgcggtaggggagactggaattcccggtgtaacggtggaatgtgtagatatcgggaagaacaccaatggcgaaggcaggtctctgggccgttactgacgctgaggagcgaaagcgtggggagcgaacaggattagataccctggtagtccacgccgtaaacggtggatgctggatgtggggcccgttccacgggttccgtgtcggagctaacgcgttaagcatcccgcctggggagtacggccgcaaggctaaaactcaaagaaattgacgggggcccgcacaagcggcggagcatgcggattaattcgatgcaacgcgaagaaccttacctgggcttgacatgttcccgacggtcgtagagatacggcttcccttcggggcgggttcacaggtggtgcatggtcgtcgtcagctcgtgtcgtgagatgttgggttaagtcccgcaacgagcgcaaccctcgccccgtgttgccagcggattatgccgggaactcacgggggaccgccggggttaactcggaggaaggtggggatgacgtcagatcatcatgccccttacgtccagggcttcacgcatgctacaatggccggtacaacgggatgcgacgcggcgacgcggagcggatccctgaaaaccggtctcagttcggatcgcagtctgcaactcgactgcgtgaaggcggagtcgctagtaatcgcgaatcagcaacgtcgcggtgaatgcgttcccgggccttgtacacaccgcccgtcaagtcatgaaagtgggcagcacccgaagccggtggcctaaccccttgtgggatggagccgtctaaggtgaggctcgtgattgggactaagtcgta

SEQ ID NO: 4 - DNA, 21 bp, Artificial Sequence
  Proteobacteria_Forward Primer
gctaacgcattaagtrycccg

SEQ ID NO: 5 - DNA, 18 bp, Artificial Sequence
  Proteobacteria_Reverse Primer
gccatgcrgcacctgtct

SEQ ID NO: 6 - DNA, 52 bp, Artificial Sequence
  Bacteria_Forward Primer
tcgtcggcagcgtcagatgtgtataagagacaggtgccagcmgccgcggtaa

SEQ ID NO: 7 - DNA, 54 bp, Artificial Sequence
  Bacteria_Reverse Primer
gtctcgtgggctcggagatgtgtataagagacagggactachvgggtwtctaat